European Patent Specification EP 3 642 360 B1, published August 16, 2023. Title: Methods and kits relating to the capture of CA-IX positive exosomes. Applicant: EXOSOMICS SIENA S.P.A. The sequence listing filed with the application follows.

SEQUENCE LISTING (32 sequences)

SEQ ID NO: 1 - DNA, 25 bp, artificial sequence
  BRAF preamp primer
taggtgattttggtctagctacagt

SEQ ID NO: 2 - DNA, 24 bp, artificial sequence
  BRAF preamp primer
ttaatcagtggaaaaatagcctca

SEQ ID NO: 3 - DNA, 25 bp, artificial sequence
  BRAF preamp primer
taggtgattttggtctagctacaga

SEQ ID NO: 4 - DNA, 24 bp, artificial sequence
  BRAF preamp primer
ttaatcagtggaaaaatagcctca

SEQ ID NO: 5 - DNA, 19 bp, artificial sequence
  KRAS preamp primer
ggtagttggagctggtggc

SEQ ID NO: 6 - DNA, 26 bp, artificial sequence
  KRAS preamp primer
tgattctgaattagctgtatcgtcaa

SEQ ID NO: 7 - DNA, 25 bp, artificial sequence
  BRAF qPCR primer or probe
taggtgattttggtctagctacagt

SEQ ID NO: 8 - DNA, 24 bp, artificial sequence
  BRAF qPCR primer or probe
ttaatcagtggaaaaatagcctca

SEQ ID NO: 9 - DNA, 25 bp, artificial sequence
  BRAF qPCR primer or probe
taggtgattttggtctagctacaga

SEQ ID NO: 10 - DNA, 24 bp, artificial sequence
  BRAF qPCR primer or probe
ttaatcagtggaaaaatagcctca

SEQ ID NO: 11 - DNA, 38 bp, artificial sequence
  BRAF qPCR primer or probe
ccgaaggggatccagacaactgttcaaactgccttcgg

SEQ ID NO: 12 - DNA, 19 bp, artificial sequence
  KRAS qPCR primer or probe
ggtagttggagctggtggc

SEQ ID NO: 13 - DNA, 26 bp, artificial sequence
  KRAS qPCR primer or probe
tgattctgaattagctgtatcgtcaa

SEQ ID NO: 14 - DNA, 15 bp, artificial sequence
  KRAS qPCR primer or probe
cactcttgcctacgc

SEQ ID NO: 15 - DNA, 23 bp, artificial sequence
  EGFR qPCR primer or probe
gcagcatgtcaagatcacagatt

SEQ ID NO: 16 - DNA, 25 bp, artificial sequence
  EGFR qPCR primer or probe
cctccttctgcatggtattctttct

SEQ ID NO: 17 - DNA, 16 bp, artificial sequence
  EGFR qPCR primer or probe
agtttggccagcccaa

SEQ ID NO: 18 - DNA, 22 bp, artificial sequence
  cMyc qPCR primer or probe
ccctccactcggaaggactatc

SEQ ID NO: 19 - DNA, 22 bp, artificial sequence
  cMyc qPCR primer or probe
aggactctgacactgtccaact

SEQ ID NO: 20 - DNA, 18 bp, artificial sequence
  cMyc qPCR primer or probe
tgaccctcttggcagcag

SEQ ID NO: 21 - DNA, 23 bp, artificial sequence
  LINE qPCR primer or probe
tcaacaagaagagctaactatcc

SEQ ID NO: 22 - DNA, 22 bp, artificial sequence
  LINE qPCR primer or probe
ttgtaggtcactcaggacttgc

SEQ ID NO: 23 - DNA, 29 bp, artificial sequence
  LINE qPCR primer or probe
tgcacccaatacaggagcacccagattca

SEQ ID NO: 24 - DNA, 24 bp, artificial sequence
  HERV-W qPCR primer or probe
cttccagaattgaagctgtaaagc

SEQ ID NO: 25 - DNA, 22 bp, artificial sequence
  HERV-W qPCR primer or probe
gggttgtgcagttgagatttcc

SEQ ID NO: 26 - DNA, 26 bp, artificial sequence
  HERV-W qPCR primer or probe
ttcttcaaatggagccccagatgcag

SEQ ID NO: 27 - DNA, 21 bp, artificial sequence
  AR-WT FW primer
cagcctattgcgagagagctg

SEQ ID NO: 28 - DNA, 21 bp, artificial sequence
  AR-WT RW primer
gaaaggatcttgggcacttgc

SEQ ID NO: 29 - DNA, 18 bp, artificial sequence
  AR-WT probe
agttcacttttgacctgc

SEQ ID NO: 30 - DNA, 26 bp, artificial sequence
  AR-V7 FW primer
ccatcttgtcgtcttcggaaatgtta

SEQ ID NO: 31 - DNA, 26 bp, artificial sequence
  AR-V7 RW primer
tttgaatgaggcaagtcagcctttct

SEQ ID NO: 32 - DNA, 17 bp, artificial sequence
  AR-V7 probe
aagcagggatgactctg